European Patent Application EP 4 659 760 A1, published December 10, 2025. Title: Therapeutic immune intervention. Applicant: Helmholtz Zentrum fuer Infektionsforschung GmbH. Application EP. The sequence listing filed with the application follows.

SEQUENCE LISTING (1 sequence)

SEQ ID NO: 1 - protein, 557 aa, synthetic construct
MAPAAVDWRARGAVTAVKDQGQCGSCWAFSAIGNVECQWFLAGHPLTNLSEQMLVSCDKTDSGCGGGLMNNAFEWIVQENNGAVYTEGSYPYASGEGISPPCTTSGHTVGATITGHVELPQDEAQIAAWLAVNGPVAVAVDASSWMTYTGGVMTSCVSEQLDHGVLLVGYNDSAAVPYWVIKNSWATQWGEDGYIRIAKGSNQCLVKEEASSAVVGLVGELRIIKSVLQSWKNWDSHLSSTDVVTAGGSGIVMQNDTPVFPLMVNGENYPFSSITYSTDKGNNWVFPEGISPVGCLDPRITEWETGQILMIVQCKDDQSVFESRDMGKTWTEAIGTLSGVWVMSQPGVRLYKIFRVGALVTATIEGRKVMLYTQRGYTSGEKEANALYLWVTDNNRTFHVGPLFLEDNVNETLANALLYSDGALHLLKERANEKDEAISLARLTEELNTIKSVLSTWAKLDASFSESSTPTAGLVGFLSNTSSGGDTWIDDYRCVHASVTKASKVKNGFKFMGPGSMATWLVNSREDNRQYSFVHHRFTIVATVTIHQVPKHHHHHH